European Patent Application EP 4 186 975 A1, published May 31, 2023. Title: Non-Integrating DNA Vectors for the genetic modification of Cells. Applicant: Deutsches Krebsforschungszentrum. Application EP. The sequence listing filed with the application follows.

SEQUENCE LISTING (15 sequences)

SEQ ID NO: 1-2 - skipped (2 entries)

SEQ ID NO: 3 - DNA, 11 bp, Homo sapiens
  source 1..11: mol_type = genomic DNA
taaatatttta

SEQ ID NO: 4 - DNA, 19 bp, Homo sapiens
  source 1..19: mol_type = genomic DNA
attataaatattttaatta

SEQ ID NO: 5 - DNA, 24 bp, Homo sapiens
  source 1..24: mol_type = genomic DNA
atttaattataaatattttaatta

SEQ ID NO: 6 - DNA, 525 bp, Homo sapiens
  source 1..525: mol_type = genomic DNA
atttataaaatattgaattataaaatatgtaattataaatactttaattataaaatatgtaattataaatactttaattataaaatatgtaattataaatactttataaaatatgtaattataaaatatgtaattataaacattttaattataaaatatgtaattataaacattttaattataaaatatgtaattataaacattttaattataaaatatgtaattataaacattttaattataaaatatgtaattataaacattttaattataaaatatttaattataaacattttaattataaaatatttaattataaatattttaattataaaatatttaattataaatattttaattataaaatatttaattataaatattttaattataaaatatttaattataaatactttaattataaaatatttaattataaatattttaattataaaatatttaattataaatattttaattataaatattttaattataaaatatttaattataaaaacacaatta

SEQ ID NO: 7 - DNA, 825 bp, Homo sapiens
  source 1..825: mol_type = genomic DNA
gcaggctgagtgaaataaaggacttgttatttcatctcgaggcctaccggagagccttgccttgcaaaggcagacagtcagtgaggaagactatgtggcacatgaagacaccagaggtgttcctcaggatcaaagtatgtacaagcctttgtgaatattttttccttctcacttggcaaatacaattcctgagatcaataacctcgtctttttaattttttcctcgtctttttaactatttataaaatattgaattataaaatatgtaattataaatactttaattataaaatatgtaattataaatactttaattataaaatatgtaattataaatactttataaaatatgtaattataaaatatgtaattataaacattttaattataaaatatgtaattataaacattttaattataaaatatgtaattataaacattttaattataaaatatgtaattataaacattttaattataaaatatgtaattataaacattttaattataaaatatttaattataaacattttaattataaaatatttaattataaatattttaattataaaatatttaattataaatattttaattataaaatatttaattataaatattttaattataaaatatttaattataaatactttaattataaaatatttaattataaatattttaattataaaatatttaattataaatattttaattataaatattttaattataaaatatttaattataaaaacacaattacctcatctttttaaatatttttgcaaaatatttccctccataatttctccgtttccattttta

SEQ ID NO: 8 - DNA, 854 bp, Homo sapiens
  source 1..854: mol_type = genomic DNA
cttctccactcctggcaggctgagtgaaataaaggacttgttatttcatctcgaggcctaccggagagccttgccttgcaaaggcagacagtcagtgaggaagactatgtggcacatgaagacaccagaggtgttcctcaggatcaaagtatgtacaagcctttgtgaatattttttccttctcacttggcaaatacaattcctgagatcaataacctcgtctttttaattttttcctcgtctttttaactatttataaaatattgaattataaaatatgtaattataaatactttaattataaaatatgtaattataaatactttaattataaaatatgtaattataaatactttataaaatatgtaattataaaatatgtaattataaacattttaattataaaatatgtaattataaacattttaattataaaatatgtaattataaacattttaattataaaatatgtaattataaacattttaattataaaatatgtaattataaacattttaattataaaatatttaattataaacattttaattataaaatatttaattataaatattttaattataaaatatttaattataaatattttaattataaaatatttaattataaatattttaattataaaatatttaattataaatactttaattataaaatatttaattataaatattttaattataaaatatttaattataaatattttaattataaatattttaattataaaatatttaattataaaaacacaattacctcatctttttaaatatttttgcaaaatatttccctccataatttctccgtttccatttttattctgttacttaaat

SEQ ID NO: 9 - protein, 199 aa, synthetic construct
  REGION 1..199: note = puromycin acetyltransferase, synthetic construct
MTEYKPTVRLATRDDVPRAVRTLAAAFADYPATRHTVDPDRHIERVTELQELFLTRVGLDIGKVWVADDGAAVAVWTTPESVEAGAVFAEIGPRMAELSGSRLAAQQQMEGLLAPHRPKEPAWFLATVGVSPDHQGKGLGSAVVLPGVEAAERAGVPAFLETSAPRNLPFYERLGFTVTADVEVPEGPRTWCMTRKPGA

SEQ ID NO: 10 - DNA, 600 bp, synthetic construct
  misc_feature 1..600: note = puromycin acetyltransferase encoding sequence, synthetic construct
  source 1..600: mol_type = other DNA
atgaccgagtacaagcccacggtgcgcctcgccacccgcgacgacgtcccccgggccgtacgcaccctcgccgccgcgttcgccgactaccccgccacgcgccacaccgtcgacccggaccgccacatcgagcgggtcaccgagctgcaagaactcttcctcacgcgcgtcgggctcgacatcggcaaggtgtgggtcgcggacgacggcgccgcggtggcggtctggaccacgccggagagcgtcgaagcgggggcggtgttcgccgagatcggcccgcgcatggccgagttgagcggttcccggctggccgcgcagcaacagatggaaggcctcctggcgccgcaccggcccaaggagcccgcgtggttcctggccaccgtcggcgtctcgcccgaccaccagggcaagggtctgggcagcgccgtcgtgctccccggagtggaggcggccgagcgcgccggggtgcccgccttcctggagacctccgcgccccgcaacctccccttctacgagcggctcggcttcaccgtcaccgccgacgtcgaggtgcccgaaggaccgcgcacctggtgcatgacccgcaagcccggtgcctga

SEQ ID NO: 11 - DNA, 1031 bp, synthetic construct
  misc_feature 1..1031: note = anti-repressive element40
  source 1..1031: mol_type = other DNA
gatcaagaaagcactccgggctccagaaggagccttccaggccagctttgagcataagctgctgatgagcagtgagtgtcttgagtagtgttcagggcagcatgttaccattcatgcttgacttctagccagtgtgacgagaggctggagtcaggtctctagagagttgagcagctccagccttagatctcccagtcttatgcggtgtgcccattcgctttgtgtctgcagtcccctggccacacccagtaacagttctgggatctatgggagtagcttccttagtgagctttcccttcaaatactttgcaaccaggtagagaagtttggagtgaaggttttgttcttcgtttcttcacaatatggatatgcatcttcttttgaaaatgttaaagtaaattacctctcttttcagatactgtcttcatgcgaacttggtatcctgtttccatcccagccttctataacccagtaacatcttttttgaaaccagtgggtgagaaagacacctggtcaggaacgcggaccacaggacaactcaggctcacccacggcatcagactaaaggcaaacaaggactctgtataaagtaccggtggcatgtgtattagtggagatgcagcctgtgctctgcagacagggagtcacacagacacttttctataatttcttaagtgctttgaatgttcaagtagaaagtctaacattaaatttgattgaacaattgtatattcatggaatattttggaacggaataccaaaaaatggcaatagtggttctttctggatggaagacaaacttttcttctttaaaataaattttattttatatatttgaggttgaccacatgaccttaaggatacatatagacagtaaactggttactacagtgaagcaaattaacatatctaccatcgtacatagttacatttttttgtgtgacaggaacagctaaaatctacgtatttaacaaaactcctaaagacaatacatttttattaactatagccctcatgatgtacattagatc

SEQ ID NO: 12 - DNA, 1438 bp, synthetic construct
  misc_feature 1..1438: note = CMV Promoter - S/MAR sequence
  source 1..1438: mol_type = other DNA
ggcattgattattgactagttattaatagtaatcaattacggggtcattagttcatagcccatatatggagttccgcgttacataacttacggtaaatggcccgcctggctgaccgcccaacgacccccgcccattgacgtcaataatgacgtatgttcccatagtaacgccaatagggactttccattgacgtcaatgggtggagtatttacggtaaactgcccacttggcagtacatcaagtgtatcatatgccaagtccgccccctattgacgtcaatgacggtaaatggcccgcctggcattatgcccagtacatgaccttacgggactttcctacttggcagtacatctacgtattagtcatcgctattaccatggtgatgcggttttggcagtacaccaatgggcgtggatagcggtttgactcacggggatttccaagtctccaccccattgacgtcaatgggagtttgttttggcaccaaaatcaacgggactttccaaaatgtcgtaataaccccgccccgttgacgcaaatgggcggtaggcgtgtacggtgggaggtctatataagcagaggtcttctccactcctggcaggctgagtgaaataaaggacttgttatttcatctcgaggcctaccggagagccttgccttgcaaaggcagacagtcagtgaggaagactatgtggcacatgaagacaccagaggtgttcctcaggatcaaagtatgtacaagcctttgtgaatattttttccttctcacttggcaaatacaattcctgagatcaataacctcgtctttttaattttttcctcgtctttttaactatttataaaatattgaattataaaatatgtaattataaatactttaattataaaatatgtaattataaatactttaattataaaatatgtaattataaatactttataaaatatgtaattataaaatatgtaattataaacattttaattataaaatatgtaattataaacattttaattataaaatatgtaattataaacattttaattataaaatatgtaattataaacattttaattataaaatatgtaattataaacattttaattataaaatatttaattataaacattttaattataaaatatttaattataaatattttaattataaaatatttaattataaatattttaattataaaatatttaattataaatattttaattataaaatatttaattataaatactttaattataaaatatttaattataaatattttaattataaaatatttaattataaatattttaattataaatattttaattataaaatatttaattataaaaacacaattacctcatctttttaaatatttttgcaaaatatttccctccataatttctccgtttccatttttattctgttacttaaat

SEQ ID NO: 13 - DNA, 2038 bp, synthetic construct
  misc_feature 1..2038: note = CMV Promoter - Puromycin - S/MAR sequence
  source 1..2038: mol_type = other DNA
ggcattgattattgactagttattaatagtaatcaattacggggtcattagttcatagcccatatatggagttccgcgttacataacttacggtaaatggcccgcctggctgaccgcccaacgacccccgcccattgacgtcaataatgacgtatgttcccatagtaacgccaatagggactttccattgacgtcaatgggtggagtatttacggtaaactgcccacttggcagtacatcaagtgtatcatatgccaagtccgccccctattgacgtcaatgacggtaaatggcccgcctggcattatgcccagtacatgaccttacgggactttcctacttggcagtacatctacgtattagtcatcgctattaccatggtgatgcggttttggcagtacaccaatgggcgtggatagcggtttgactcacggggatttccaagtctccaccccattgacgtcaatgggagtttgttttggcaccaaaatcaacgggactttccaaaatgtcgtaataaccccgccccgttgacgcaaatgggcggtaggcgtgtacggtgggaggtctatataagcagaggtatgaccgagtacaagcccacggtgcgcctcgccacccgcgacgacgtcccccgggccgtacgcaccctcgccgccgcgttcgccgactaccccgccacgcgccacaccgtcgacccggaccgccacatcgagcgggtcaccgagctgcaagaactcttcctcacgcgcgtcgggctcgacatcggcaaggtgtgggtcgcggacgacggcgccgcggtggcggtctggaccacgccggagagcgtcgaagcgggggcggtgttcgccgagatcggcccgcgcatggccgagttgagcggttcccggctggccgcgcagcaacagatggaaggcctcctggcgccgcaccggcccaaggagcccgcgtggttcctggccaccgtcggcgtctcgcccgaccaccagggcaagggtctgggcagcgccgtcgtgctccccggagtggaggcggccgagcgcgccggggtgcccgccttcctggagacctccgcgccccgcaacctccccttctacgagcggctcggcttcaccgtcaccgccgacgtcgaggtgcccgaaggaccgcgcacctggtgcatgacccgcaagcccggtgcctgacttctccactcctggcaggctgagtgaaataaaggacttgttatttcatctcgaggcctaccggagagccttgccttgcaaaggcagacagtcagtgaggaagactatgtggcacatgaagacaccagaggtgttcctcaggatcaaagtatgtacaagcctttgtgaatattttttccttctcacttggcaaatacaattcctgagatcaataacctcgtctttttaattttttcctcgtctttttaactatttataaaatattgaattataaaatatgtaattataaatactttaattataaaatatgtaattataaatactttaattataaaatatgtaattataaatactttataaaatatgtaattataaaatatgtaattataaacattttaattataaaatatgtaattataaacattttaattataaaatatgtaattataaacattttaattataaaatatgtaattataaacattttaattataaaatatgtaattataaacattttaattataaaatatttaattataaacattttaattataaaatatttaattataaatattttaattataaaatatttaattataaatattttaattataaaatatttaattataaatattttaattataaaatatttaattataaatactttaattataaaatatttaattataaatattttaattataaaatatttaattataaatattttaattataaatattttaattataaaatatttaattataaaaacacaattacctcatctttttaaatatttttgcaaaatatttccctccataatttctccgtttccatttttattctgttacttaaat

SEQ ID NO: 14 - DNA, 6189 bp, synthetic construct
  misc_feature 1..6189: note = Element40-GPF-P2A-Puromycin-S/MAR
  source 1..6189: mol_type = other DNA
ggcattgattattgactagttattaatagtaatcaattacggggtcattagttcatagcccatatatggagttccgcgttacataacttacggtaaatggcccgcctggctgaccgcccaacgacccccgcccattgacgtcaataatgacgtatgttcccatagtaacgccaatagggactttccattgacgtcaatgggtggagtatttacggtaaactgcccacttggcagtacatcaagtgtatcatatgccaagtccgccccctattgacgtcaatgacggtaaatggcccgcctggcattatgcccagtacatgaccttacgggactttcctacttggcagtacatctacgtattagtcatcgctattaccatggtgatgcggttttggcagtacaccaatgggcgtggatagcggtttgactcacggggatttccaagtctccaccccattgacgtcaatgggagtttgttttggcaccaaaatcaacgggactttccaaaatgtcgtaataaccccgccccgttgacgcaaatgggcggtaggcgtgtacggtgggaggtctatataagcagaggtcgtttagtgaaccgtcagatcactagtagctttattgcggtagtttatcacagttaaattgctaacgcagtcagtgctcgactgatcacaggtaagtatcaaggttacaagacaggtttaaggaggccaatagaaactgggcttgtcgagacagagaagattcttgcgtttctgataggcacctattggtcttactgacatccactttgcctttctctccacaggggtaccgaagccgctagcgctaccggtcgccaccatgcccgccatgaagatcgagtgccgcatcaccggcaccctgaacggcgtggagttcgagctggtgggcggcggagagggcacccccgagcagggccgcatgaccaacaagatgaagagcaccaaaggcgccctgaccttcagcccctacctgctgagccacgtgatgggctacggcttctaccacttcggcacctaccccagcggctacgagaaccccttcctgcacgccatcaacaacggcggctacaccaacacccgcatcgagaagtacgaggacggcggcgtgctgcacgtgagcttcagctaccgctacgaggccggccgcgtgatcggcgacttcaaggtggtgggcaccggcttccccgaggacagcgtgatcttcaccgacaagatcatccgcagcaacgccaccgtggagcacctgcaccccatgggcgataacgtgctggtgggcagcttcgcccgcaccttcagcctgcgcgacggcggctactacagcttcgtggtggacagccacatgcacttcaagagcgccatccaccccagcatcctgcagaacgggggccccatgttcgccttccgccgcgtggaggagctgcacagcaacaccgagctgggcatcgtggagtaccagcacgccttcaagacccccatcgccttcgccagatctggcagcggcgccaccaacttcagcctgctgaagcaggccggcgacgtggaggaaaaccctgggcccatgaccgagtacaagcccacggtgcgcctcgccacccgcgacgacgtcccccgggccgtacgcaccctcgccgccgcgttcgccgactaccccgccacgcgccacaccgtcgacccggaccgccacatcgagcgggtcaccgagctgcaagaactcttcctcacgcgcgtcgggctcgacatcggcaaggtgtgggtcgcggacgacggcgccgcggtggcggtctggaccacgccggagagcgtcgaagcgggggcggtgttcgccgagatcggcccgcgcatggccgagttgagcggttcccggctggccgcgcagcaacagatggaaggcctcctggcgccgcaccggcccaaggagcccgcgtggttcctggccaccgtcggcgtctcgcccgaccaccagggcaagggtctgggcagcgccgtcgtgctccccggagtggaggcggccgagcgcgccggggtgcccgccttcctggagacctccgcgccccgcaacctccccttctacgagcggctcggcttcaccgtcaccgccgacgtcgaggtgcccgaaggaccgcgcacctggtgcatgacccgcaagcccggtgcctgaagatctatgcatgcagaagttggtcgtgaggcactgggcaggtaagtatcaaggttacaagacaggtcgacttctccactcctggcaggctgagtgaaataaaggacttgttatttcatctcgaggcctaccggagagccttgccttgcaaaggcagacagtcagtgaggaagactatgtggcacatgaagacaccagaggtgttcctcaggatcaaagtatgtacaagcctttgtgaatattttttccttctcacttggcaaatacaattcctgagatcaataacctcgtctttttaattttttcctcgtctttttaactatttataaaatattgaattataaaatatgtaattataaatactttaattataaaatatgtaattataaatactttaattataaaatatgtaattataaatactttataaaatatgtaattataaaatatgtaattataaacattttaattataaaatatgtaattataaacattttaattataaaatatgtaattataaacattttaattataaaatatgtaattataaacattttaattataaaatatgtaattataaacattttaattataaaatatttaattataaacattttaattataaaatatttaattataaatattttaattataaaatatttaattataaatattttaattataaaatatttaattataaatattttaattataaaatatttaattataaatactttaattataaaatatttaattataaatattttaattataaaatatttaattataaatattttaattataaatattttaattataaaatatttaattataaaaacacaattacctcatctttttaaatatttttgcaaaatatttccctccataatttctccgtttccatttttattctgttacttaaataattctgcagtcgacggttactgacatccactttgcctttctctccacaggtgtccactctaccgcgggcccgggatccaccggatctagataactgatcataatcagccataccacatttgtagaggttttacttgctttaaaaaacctcccacacctccccctgaacctgaaacataaaatgaatgcaattgttgttgttaacttgtttattgcagcttataatggttacaaataaagcaatagcatcacaaatttcacaaataaagcatttttttcactgcattctagttgtggtttgtccaaactcatcaatgtatcttacatgtgagcaaaaggccagcaaaaggccaggaaccgtaaaaaggccgcgttgctggcgtttttccataggctccgcccccctgacgagcatcacaaaaatcgacgctcaagtcagaggtggcgaaacccgacaggactataaagataccaggcgtttccccctggaagctccctcgtgcgctctcctgttccgaccctgccgcttacgggatacctgtccgcctttctcccttcgggaagcgtggcgctttctcatagctcacgctgtaggtatctcagttcggtgtaggtcgttcgctccaagctgggctgtgtgcacgaaccccccgttcagcccgaccgctgcgccttatccggtaactatcgtcttgagtccaacccggtaagacacgacttatcgccactggcagcagccactggtaacaggattagcagagcgaggtatgtaggcggtgctacagagttcttgaagtggtggcctaactacggctacactagaagaacagtatttggtatctgcgctctgctgaagccagttaccttcggaaaaagagttggtagctcttgatccggcaaacaaaccaccgctggtagcggtggtttttttgtttgcaagcagcagattacgcgcagaaaaaaaggatctcaagaagatcctttgatcttttctacggggtctgacgctcagtggaacgaaaactcacgttaagggattttggtcatgccgtctcagaagaactcgtcaagaaggcgatagaaggcgatgcgctgcgaatcgggagcggcgataccgtaaagcacgaggaagcggtcagcccattcgccgccaagctcttcagcaatatcacgggtagccaacgctatgtcctgatagcggtccgccacacccagccggccacagtcgatgaatccagaaaagcggccattttccaccatgatattcggcaagcaggcatcgccatgggtcacgacgagatcctcgccgtcgggcatgctcgccttgagcctggcgaacagttcggctggcgcgagcccctgatgctcttcgtccagatcatcctgatcgacaagaccggcttccatccgagtacgtgctctctcgatgcgatgtttcgcttggtggtcgaatgggcaggtagccggatcaagcgtatgcagccgccgcattgcatcagccatgatggatactttctcggcaggagcaaggtgagatgacaggagatcctgccccggcacttcgcccaatagcagccagtcccttcccgcttcagtgacaacgtcgagtacagctgcgcaaggaacgcccgtcgtggccagccacgatagccgcgctgcctcgtcttgcagttcattcagggcaccggacaggtcggtcttgacaaaaagaaccgggcgcccctgcgctgacagccggaacacggcggcatcagagcagccgattgtctgttgtgcccagtcatagccgaatagcctctccacccaagcggccggagaacctgcgtgcaatccatcttgttcaatcataatattattgaagcatttatcagggttcgtctcgtcccggtctcctcccatgcatgtcaatattggccattagccatattattcattggttatatagcataaatcaatattggctattggccattgcatacgttgtatctatatcataatatgtacaaagcttgatcaagaaagcactccgggctccagaaggagccttccaggccagctttgagcataagctgctgatgagcagtgagtgtcttgagtagtgttcagggcagcatgttaccattcatgcttgacttctagccagtgtgacgagaggctggagtcaggtctctagagagttgagcagctccagccttagatctcccagtcttatgcggtgtgcccattcgctttgtgtctgcagtcccctggccacacccagtaacagttctgggatctatgggagtagcttccttagtgagctttcccttcaaatactttgcaaccaggtagagaagtttggagtgaaggttttgttcttcgtttcttcacaatatggatatgcatcttcttttgaaaatgttaaagtaaattacctctcttttcagatactgtcttcatgcgaacttggtatcctgtttccatcccagccttctataacccagtaacatcttttttgaaaccagtgggtgagaaagacacctggtcaggaacgcggaccacaggacaactcaggctcacccacggcatcagactaaaggcaaacaaggactctgtataaagtaccggtggcatgtgtattagtggagatgcagcctgtgctctgcagacagggagtcacacagacacttttctataatttcttaagtgctttgaatgttcaagtagaaagtctaacattaaatttgattgaacaattgtatattcatggaatattttggaacggaataccaaaaaatggcaatagtggttctttctggatggaagacaaacttttcttctttaaaataaattttattttatatatttgaggttgaccacatgaccttaaggatacatatagacagtaaactggttactacagtgaagcaaattaacatatctaccatcgtacatagttacatttttttgtgtgacaggaacagctaaaatctacgtatttaacaaaactcctaaagacaatacatttttattaactatagccctcatgatgtacattagatctgtacatttatattggctcatgtccaatatgaccgccatgtt

SEQ ID NO: 15 - DNA, 248 bp, Homo sapiens
  source 1..248: mol_type = genomic DNA
atttaattataaacattttaattataaaatatttaattataaatattttaattataaaatatttaattataaatattttaattataaaatatttaattataaatattttaattataaaatatttaattataaatactttaattataaaatatttaattataaatattttaattataaaatatttaattataaatattttaattataaatattttaattataaaatatttaattataaaaacacaatta